European Patent Specification EP 3 861 134 B1, published September 4, 2024. Title: DETERMINING 5' TRANSCRIPT SEQUENCES. Applicant: CELLULAR RESEARCH, INC. CHANG, Christina SHUM, Eleen. The sequence listing filed with the application follows.

SEQUENCE LISTING (1 sequence)

SEQ ID NO: 1 - DNA, 21 bp, Artificial Sequence
  Template Switch Oligonucleotide
  misc_feature (19)..(21): n is riboguanosine
ttttttttttttttttttnnn